European Patent Specification EP 4 469 042 B1, published August 26, 2026. Title: A GluN2D inhibitor or a mGluR2 inhibitor for use in the treatment or relapse prevention of a depressive episode. Applicant: Albert-Ludwigs-Universität Freiburg. The sequence listing filed with the application follows.

SEQUENCE LISTING (10 sequences)

SEQ ID NO: 1 - RNA, 21 nt, synthetic construct
  source 1..21: mol_type = other RNA
  modified_base 20: mod_base = OTHER; note = thymine
  modified_base 21: mod_base = OTHER; note = thymine
gcaactatcccgacatgcatt

SEQ ID NO: 2 - RNA, 21 nt, synthetic construct
  source 1..21: mol_type = other RNA
tgcatgtcgggatagttgctg

SEQ ID NO: 3 - RNA, 21 nt, synthetic construct
  source 1..21: mol_type = other RNA
  modified_base 20: mod_base = OTHER; note = thymine
  modified_base 21: mod_base = OTHER; note = thymine
gcaactatcccgacatgcatt

SEQ ID NO: 4 - RNA, 21 nt, synthetic construct
  source 1..21: mol_type = other RNA
tgatctttgactcctgttcaa

SEQ ID NO: 5 - DNA, 22 bp, synthetic construct
  misc_feature 1..22: note = synthetic
  source 1..22: mol_type = other DNA
ctgtgtgggtgatgatgttcgt

SEQ ID NO: 6 - DNA, 20 bp, synthetic construct
  misc_feature 1..20: note = synthetic
  source 1..20: mol_type = other DNA
gtgaaggtagagcctccggg

SEQ ID NO: 7 - DNA, 22 bp, synthetic construct
  misc_feature 1..22: note = synthetic
  source 1..22: mol_type = other DNA
acaactttggtatcgtggaagg

SEQ ID NO: 8 - DNA, 19 bp, synthetic construct
  misc_feature 1..19: note = synthetic
  source 1..19: mol_type = other DNA
gccatcacgccacagtttc

SEQ ID NO: 9 - DNA, 20 bp, synthetic construct
  misc_feature 1..20: note = synthetic
  source 1..20: mol_type = other DNA
gcggcggaaaatagcctttg

SEQ ID NO: 10 - DNA, 21 bp, synthetic construct
  misc_feature 1..21: note = synthetic
  source 1..21: mol_type = other DNA
gatcacacgttccacctcatc